European Patent Application EP 4 745 153 A1, published May 20, 2026. Title: GLP-1, GIP AND GCG RECEPTOR TRIAGONIST AND USE THEREOF. Applicant: BEIJING TUO JIE BIOPHARMACEUTICAL CO., LTD. The sequence listing filed with the application follows.

SEQUENCE LISTING (151 sequences)

SEQ ID NO: 1 - protein, 39 aa, synthetic construct
  SITE 2: note = X is Aib
  SITE 12: note = K is alpha-methyl-Lys
  MOD_RES 39: note = The C-terminal Ser is amidated
HXHGTFTSDYSKYLEEKAAQEFVEWLLAGGPSSGAPPPS

SEQ ID NO: 2 - protein, 39 aa, synthetic construct
  SITE 2: note = X is Aib
  SITE 12: note = K is alpha-methyl-Lys
  MOD_RES 39: note = The C-terminal Ser is amidated
HXHGTFTSDYSKYLEKKAAQEFVEWLLAGGPSSGAPPPS

SEQ ID NO: 3 - protein, 39 aa, synthetic construct; identical to SEQ ID NO: 2
  SITE 2: note = X is Aib
  SITE 13: note = Y is alpha-methyl-Tyr
  MOD_RES 39: note = The C-terminal Ser is amidated

SEQ ID NO: 4 - protein, 39 aa, synthetic construct
  SITE 2: note = X is Aib
  SITE 13: note = X is Aib
  MOD_RES 39: note = The C-terminal Ser is amidated
HXHGTFTSDYSKXLEKKAAQEFVEWLLAGGPSSGAPPPS

SEQ ID NO: 5 - protein, 39 aa, synthetic construct; identical to SEQ ID NO: 2
  SITE 2: note = X is Aib
  SITE 14: note = L is alpha-methyl-Leu
  MOD_RES 39: note = The C-terminal Ser is amidated

SEQ ID NO: 6 - protein, 39 aa, synthetic construct; identical to SEQ ID NO: 2
  SITE 2: note = X is Aib
  SITE 17: note = K is alpha-methyl-Lys
  MOD_RES 39: note = The C-terminal Ser is amidated

SEQ ID NO: 7 - protein, 39 aa, synthetic construct
  SITE 2: note = X is Aib
  SITE 18: note = X is Aib
  MOD_RES 39: note = The C-terminal Ser is amidated
HXHGTFTSDYSKYLEKKXAQEFVEWLLAGGPSSGAPPPS

SEQ ID NO: 8 - protein, 39 aa, synthetic construct
  SITE 2: note = X is Aib
  MOD_RES 39: note = The C-terminal Ser is amidated
  SITE 12: note = K is alpha-methyl-Lys
HXHGTFTSDYSKYLEKKAAQEFVEWLIAGGPSSGAPPPS

SEQ ID NO: 9 - protein, 39 aa, synthetic construct
  SITE 2: note = X is Aib
  MOD_RES 39: note = The C-terminal Ser is amidated
  SITE 12: note = K is alpha-methyl-Lys
HXHGTFTSDYSKLLEKKAAQEFVEWLLAGGPSSGAPPPS

SEQ ID NO: 10 - protein, 39 aa, synthetic construct
  SITE 2: note = X is Aib
  MOD_RES 39: note = The C-terminal Ser is amidated
  SITE 12: note = K is alpha-methyl-Lys
HXHGTFTSDYSKYLEKKAQQEFVEWLLAGGPSSGAPPPS

SEQ ID NO: 11 - protein, 39 aa, synthetic construct
  SITE 2: note = X is Aib
  MOD_RES 39: note = The C-terminal Ser is amidated
  SITE 12: note = K is alpha-methyl-Lys
YXQGTFTSDYSKLLEKKAAQEFVEWLLAGGPSSGAPPPS

SEQ ID NO: 12 - protein, 39 aa, synthetic construct
  SITE 2: note = X is Aib
  MOD_RES 39: note = The C-terminal Ser is amidated
  SITE 12: note = K is alpha-methyl-Lys
HXHGTFTSDYSKYLEKKAAQEFVEWLIEGGPSSGAPPPS

SEQ ID NO: 13 - protein, 39 aa, synthetic construct
  SITE 2: note = X is Aib
  MOD_RES 39: note = The C-terminal Ser is amidated
  SITE 12: note = K is alpha-methyl-Lys
HXHGTFTSDYSKLLEKQAAQEFVEWLLAGGPSSGAPPPS

SEQ ID NO: 14 - protein, 39 aa, synthetic construct
  SITE 2: note = X is Aib
  MOD_RES 39: note = The C-terminal Ser is amidated
  SITE 12: note = K is alpha-methyl-Lys
HXHGTFTSDYSKLLEKIAAQEFVEWLLAGGPSSGAPPPS

SEQ ID NO: 15 - protein, 39 aa, synthetic construct
  SITE 2: note = X is Aib
  MOD_RES 39: note = The C-terminal Ser is amidated
  SITE 12: note = K is alpha-methyl-Lys
HXHGTFTSDYSKILEKKAAQEFVEWLLAGGPSSGAPPPS

SEQ ID NO: 16 - protein, 39 aa, synthetic construct
  SITE 2: note = X is Aib
  MOD_RES 39: note = The C-terminal Ser is amidated
HXHGTFTSDYSILLEKKAAQEFVEWLLAGGPSSGAPPPS

SEQ ID NO: 17 - protein, 39 aa, synthetic construct; identical to SEQ ID NO: 16
  SITE 2: note = X is Aib
  MOD_RES 39: note = The C-terminal Ser is amidated
  SITE 13: note = L is alpha-methyl-Leu

SEQ ID NO: 18 - protein, 39 aa, synthetic construct
  SITE 2: note = X is Aib
  MOD_RES 39: note = The C-terminal Ser is amidated
  SITE 12: note = K is alpha-methyl-Lys
  SITE 20: note = S is alpha-methyl-Ser
HXHGTFTSDYSKLLEKKAASEFVEWLIEGGPSSGAPPPS

SEQ ID NO: 19 - protein, 39 aa, synthetic construct
  SITE 2: note = X is Aib
  MOD_RES 39: note = The C-terminal Ser is amidated
  SITE 12: note = K is alpha-methyl-Lys
  SITE 20: note = X is isovaline
YXQGTFTSDYSKLLEKKAAXEFVEWLLAGGPSSGAPPPS

SEQ ID NO: 20 - protein, 39 aa, synthetic construct
  SITE 2: note = X is Aib
  MOD_RES 39: note = The C-terminal Ser is amidated
  SITE 12: note = K is alpha-methyl-Lys
  SITE 20: note = X is isovaline
HXHGTFTSDYSKLLEKQAAXEFVEWLLAGGPSSGAPPPS

SEQ ID NO: 21 - protein, 39 aa, synthetic construct
  SITE 2: note = X is Aib
  MOD_RES 39: note = The C-terminal Ser is amidated
  SITE 12: note = K is alpha-methyl-Lys
  SITE 20: note = X is isovaline
YXQGTFTSDYSKILEKKAAXEFVEWLLAGGPSSGAPPPS

SEQ ID NO: 22 - protein, 39 aa, synthetic construct
  SITE 2: note = X is Aib
  MOD_RES 39: note = The C-terminal Ser is amidated
  SITE 12: note = K is alpha-methyl-Lys
  SITE 20: note = X is isovaline
HXHGTFTSDYSKILEKQAAXEFVEWLLAGGPSSGAPPPS

SEQ ID NO: 23 - protein, 39 aa, synthetic construct
  SITE 2: note = X is Aib
  MOD_RES 39: note = The C-terminal Ser is amidated
  SITE 12: note = K is alpha-methyl-Lys
  SITE 20: note = X is isovaline
HXHGTFTSDYSKLLEKKAAXEFVEWLIEGGPSSGAPPPS

SEQ ID NO: 24 - protein, 39 aa, synthetic construct
  SITE 2: note = X is Aib
  MOD_RES 39: note = The C-terminal Ser is amidated
  SITE 12: note = K is alpha-methyl-Lys
  SITE 20: note = X is isovaline
HXHGTFTSDYSKILEKKAAXEFVEWLIEGGPSSGAPPPS

SEQ ID NO: 25 - protein, 39 aa, synthetic construct
  SITE 2: note = X is Aib
  MOD_RES 39: note = The C-terminal Ser is amidated
  SITE 12: note = K is alpha-methyl-Lys
  SITE 20: note = X is isovaline
HXHGTFTSDLSKLLEKKAAXEFVEWLIEGGPSSGAPPPS

SEQ ID NO: 26 - protein, 39 aa, synthetic construct
  SITE 2: note = X is Aib
  MOD_RES 39: note = The C-terminal Ser is amidated
  SITE 12: note = K is alpha-methyl-Lys
  SITE 20: note = X is isovaline
HXHGTFTSDLSKILEKKAAXEFVEWLIEGGPSSGAPPPS

SEQ ID NO: 27 - protein, 39 aa, synthetic construct
  SITE 2: note = X is Aib
  MOD_RES 39: note = The C-terminal Ser is amidated
  SITE 20: note = X is isovaline
HXHGTFTSDYSILLEKKAAXEFVEWLLAGGPSSGAPPPS

SEQ ID NO: 28 - protein, 39 aa, synthetic construct
  SITE 2: note = X is Aib
  MOD_RES 39: note = The C-terminal Ser is amidated
  SITE 20: note = X is isovaline
HXHGTFTSDLSILLEKKAAXEFVEWLLAGGPSSGAPPPS

SEQ ID NO: 29 - protein, 39 aa, synthetic construct; identical to SEQ ID NO: 27
  SITE 2: note = X is Aib
  MOD_RES 39: note = The C-terminal Ser is amidated
  SITE 13: note = L is alpha-methyl-Leu
  SITE 20: note = X is isovaline

SEQ ID NO: 30 - protein, 39 aa, synthetic construct; identical to SEQ ID NO: 28
  SITE 2: note = X is Aib
  MOD_RES 39: note = The C-terminal Ser is amidated
  SITE 13: note = L is alpha-methyl-Leu
  SITE 20: note = X is isovaline

SEQ ID NO: 31 - protein, 39 aa, synthetic construct
  SITE 2: note = X is Aib
  MOD_RES 39: note = The C-terminal Ser is amidated
  SITE 13: note = L is alpha-methyl-Leu
  SITE 29: note = E is D-Glu
HXHGTFTSDYSILLEKKAAQEFVEWLLAEGPSSGAPPPS

SEQ ID NO: 32 - protein, 39 aa, synthetic construct; identical to SEQ ID NO: 28
  SITE 2: note = X is Aib
  MOD_RES 39: note = The C-terminal Ser is amidated
  SITE 13: note = L is alpha-methyl-Leu
  SITE 20: note = X is 1-aminocyclobutane-1-carboxylic acid

SEQ ID NO: 33 - protein, 39 aa, synthetic construct
  SITE 2: note = X is Aib
  MOD_RES 39: note = The C-terminal Ser is amidated
  SITE 13: note = L is alpha-methyl-Leu
  SITE 29: note = E is D-Glu
HXHGTFTSDLSILLEKKAAQEFVEWLLAEGPSSGAPPPS

SEQ ID NO: 34 - protein, 39 aa, synthetic construct
  SITE 2: note = X is Aib
  MOD_RES 39: note = The C-terminal Ser is amidated
  SITE 13: note = L is alpha-methyl-Leu
HXHGTFTSDLSILLEKKAAQEFVEWLLAGGPSSGAPPPS

SEQ ID NO: 35 - protein, 39 aa, synthetic construct; identical to SEQ ID NO: 33
  SITE 2: note = X is Aib
  MOD_RES 39: note = The C-terminal Ser is amidated
  SITE 29: note = E is D-Glu

SEQ ID NO: 36 - protein, 39 aa, synthetic construct
  SITE 2: note = X is Aib
  MOD_RES 39: note = The C-terminal Ser is amidated
  SITE 20: note = X is 1-aminocyclobutane-1-carboxylic acid
  SITE 29: note = E is D-Glu
HXHGTFTSDLSILLEKQAAXEFVEWLLAEGPSSGAPPPS

SEQ ID NO: 37 - protein, 39 aa, synthetic construct
  SITE 2: note = X is Aib
  MOD_RES 39: note = The C-terminal Ser is amidated
  SITE 20: note = X is 1-aminocyclopropane-1-carboxylic acid
  SITE 29: note = E is D-Glu
HXHGTFTSDLSILLEKKAAXEFVEWLLAEGPSSGAPPPS

SEQ ID NO: 38 - protein, 39 aa, synthetic construct; identical to SEQ ID NO: 37
  SITE 2: note = X is Aib
  MOD_RES 39: note = The C-terminal Ser is amidated
  SITE 20: note = X is 1-aminocyclobutane-1-carboxylic acid
  SITE 29: note = E is D-Glu

SEQ ID NO: 39 - protein, 39 aa, synthetic construct; identical to SEQ ID NO: 36
  SITE 2: note = X is Aib
  MOD_RES 39: note = The C-terminal Ser is amidated
  SITE 20: note = X is 1-aminocyclopropane-1-carboxylic acid
  SITE 29: note = E is D-Glu

SEQ ID NO: 40 - protein, 39 aa, synthetic construct
  SITE 2: note = X is Aib
  MOD_RES 39: note = The C-terminal Ser is amidated
  SITE 20: note = X is 1-aminocyclopropane-1-carboxylic acid
  SITE 29: note = E is D-Glu
HXHGTFTSDYSILLEKQAAXEFVEWLLAEGPSSGAPPPS

SEQ ID NO: 41 - protein, 39 aa, synthetic construct; identical to SEQ ID NO: 40
  SITE 2: note = X is Aib
  MOD_RES 39: note = The C-terminal Ser is amidated
  SITE 20: note = X is 1-aminocyclobutane-1-carboxylic acid
  SITE 29: note = E is D-Glu

SEQ ID NO: 42 - protein, 39 aa, synthetic construct; identical to SEQ ID NO: 31
  SITE 2: note = X is Aib
  MOD_RES 39: note = The C-terminal Ser is amidated
  SITE 29: note = E is D-Glu

SEQ ID NO: 43 - protein, 39 aa, synthetic construct
  SITE 2: note = X is Aib
  MOD_RES 39: note = The C-terminal Ser is amidated
HXHGTFTSDYSILLEKQAAQEFVEWLLAGGPSSGAPPPS

SEQ ID NO: 44 - protein, 39 aa, synthetic construct
  SITE 2: note = X is Aib
  MOD_RES 39: note = The C-terminal Ser is amidated
  SITE 29: note = E is D-Glu
HXHGTFTSDYSILLEKQAAQEFVEWLLAEGPSSGAPPPS

SEQ ID NO: 45 - protein, 39 aa, synthetic construct
  SITE 2: note = X is Aib
  MOD_RES 39: note = The C-terminal Ser is amidated
HXQGTFTSDYSILLEKKAAQEFVEWLLAGGPSSGAPPPS

SEQ ID NO: 46 - protein, 39 aa, synthetic construct; identical to SEQ ID NO: 45
  SITE 2: note = X is Aib
  MOD_RES 39: note = The C-terminal Ser is amidated
  SITE 13: note = L is alpha-methyl-Leu

SEQ ID NO: 47 - protein, 39 aa, synthetic construct
  SITE 2: note = X is Aib
  MOD_RES 39: note = The C-terminal Ser is amidated
  SITE 20: note = X is Aib
HXQGTFTSDYSILLEKKAAXEFVEWLLAGGPSSGAPPPS

SEQ ID NO: 48 - protein, 39 aa, synthetic construct; identical to SEQ ID NO: 47
  SITE 2: note = X is Aib
  MOD_RES 39: note = The C-terminal Ser is amidated
  SITE 13: note = L is alpha-methyl-Leu
  SITE 20: note = X is Aib

SEQ ID NO: 49 - protein, 39 aa, synthetic construct
  SITE 2: note = X is Aib
  SITE 12: note = K is alpha-methyl-Lys
  MOD_RES 39: note = The C-terminal Ser is amidated
  SITE 17: note = X is a Lys, Orn, Dap, Dab, or Cys residue with the side chain linked to a substituent
HXHGTFTSDYSKYLEEXAAQEFVEWLLAGGPSSGAPPPS

SEQ ID NO: 50 - protein, 39 aa, synthetic construct
  SITE 2: note = X is Aib
  SITE 12: note = K is alpha-methyl-Lys
  MOD_RES 39: note = The C-terminal Ser is amidated
  SITE 16: note = X is a Lys, Orn, Dap, Dab, or Cys residue with the side chain linked to a substituent
HXHGTFTSDYSKYLEXKAAQEFVEWLLAGGPSSGAPPPS

SEQ ID NO: 51 - protein, 39 aa, synthetic construct; identical to SEQ ID NO: 50
  SITE 2: note = X is Aib
  SITE 13: note = Y is alpha-methyl-Tyr
  MOD_RES 39: note = The C-terminal Ser is amidated
  SITE 16: note = X is a Lys, Orn, Dap, Dab, or Cys residue with the side chain linked to a substituent

SEQ ID NO: 52 - protein, 39 aa, synthetic construct
  SITE 2: note = X is Aib
  SITE 13: note = X is Aib
  MOD_RES 39: note = The C-terminal Ser is amidated
  SITE 16: note = X is a Lys, Orn, Dap, Dab, or Cys residue with the side chain linked to a substituent
HXHGTFTSDYSKXLEXKAAQEFVEWLLAGGPSSGAPPPS

SEQ ID NO: 53 - protein, 39 aa, synthetic construct; identical to SEQ ID NO: 50
  SITE 2: note = X is Aib
  SITE 14: note = L is alpha-methyl-Leu
  MOD_RES 39: note = The C-terminal Ser is amidated
  SITE 16: note = X is a Lys, Orn, Dap, Dab, or Cys residue with the side chain linked to a substituent

SEQ ID NO: 54 - protein, 39 aa, synthetic construct; identical to SEQ ID NO: 50
  SITE 2: note = X is Aib
  SITE 17: note = K is alpha-methyl-Lys
  MOD_RES 39: note = The C-terminal Ser is amidated
  SITE 16: note = X is a Lys, Orn, Dap, Dab, or Cys residue with the side chain linked to a substituent

SEQ ID NO: 55 - protein, 39 aa, synthetic construct
  SITE 2: note = X is Aib
  SITE 18: note = X is Aib
  MOD_RES 39: note = The C-terminal Ser is amidated
  SITE 16: note = X is a Lys, Orn, Dap, Dab, or Cys residue with the side chain linked to a substituent
HXHGTFTSDYSKYLEXKXAQEFVEWLLAGGPSSGAPPPS

SEQ ID NO: 56 - protein, 39 aa, synthetic construct
  SITE 2: note = X is Aib
  MOD_RES 39: note = The C-terminal Ser is amidated
  SITE 12: note = K is alpha-methyl-Lys
  SITE 16: note = X is a Lys, Orn, Dap, Dab, or Cys residue with the side chain linked to a substituent
HXHGTFTSDYSKYLEXKAAQEFVEWLIAGGPSSGAPPPS

SEQ ID NO: 57 - protein, 39 aa, synthetic construct
  SITE 2: note = X is Aib
  MOD_RES 39: note = The C-terminal Ser is amidated
  SITE 12: note = K is alpha-methyl-Lys
  SITE 16: note = X is a Lys, Orn, Dap, Dab, or Cys residue with the side chain linked to a substituent
HXHGTFTSDYSKLLEXKAAQEFVEWLLAGGPSSGAPPPS

SEQ ID NO: 58 - protein, 39 aa, synthetic construct
  SITE 2: note = X is Aib
  MOD_RES 39: note = The C-terminal Ser is amidated
  SITE 12: note = K is alpha-methyl-Lys
  SITE 16: note = X is a Lys, Orn, Dap, Dab, or Cys residue with the side chain linked to a substituent
HXHGTFTSDYSKYLEXKAQQEFVEWLLAGGPSSGAPPPS

SEQ ID NO: 59 - protein, 39 aa, synthetic construct
  SITE 2: note = X is Aib
  MOD_RES 39: note = The C-terminal Ser is amidated
  SITE 12: note = K is alpha-methyl-Lys
  SITE 16: note = X is a Lys, Orn, Dap, Dab, or Cys residue with the side chain linked to a substituent
YXQGTFTSDYSKLLEXKAAQEFVEWLLAGGPSSGAPPPS

SEQ ID NO: 60 - protein, 39 aa, synthetic construct
  SITE 2: note = X is Aib
  MOD_RES 39: note = The C-terminal Ser is amidated
  SITE 12: note = K is alpha-methyl-Lys
  SITE 16: note = X is a Lys, Orn, Dap, Dab, or Cys residue with the side chain linked to a substituent
HXHGTFTSDYSKYLEXKAAQEFVEWLIEGGPSSGAPPPS

SEQ ID NO: 61 - protein, 39 aa, synthetic construct
  SITE 2: note = X is Aib
  MOD_RES 39: note = The C-terminal Ser is amidated
  SITE 12: note = K is alpha-methyl-Lys
  SITE 16: note = X is a Lys, Orn, Dap, Dab, or Cys residue with the side chain linked to a substituent
HXHGTFTSDYSKLLEXQAAQEFVEWLLAGGPSSGAPPPS

SEQ ID NO: 62 - protein, 39 aa, synthetic construct
  SITE 2: note = X is Aib
  MOD_RES 39: note = The C-terminal Ser is amidated
  SITE 12: note = K is alpha-methyl-Lys
  SITE 16: note = X is a Lys, Orn, Dap, Dab, or Cys residue with the side chain linked to a substituent
HXHGTFTSDYSKLLEXIAAQEFVEWLLAGGPSSGAPPPS

SEQ ID NO: 63 - protein, 39 aa, synthetic construct
  SITE 2: note = X is Aib
  MOD_RES 39: note = The C-terminal Ser is amidated
  SITE 12: note = K is alpha-methyl-Lys
  SITE 16: note = X is a Lys, Orn, Dap, Dab, or Cys residue with the side chain linked to a substituent
HXHGTFTSDYSKILEXKAAQEFVEWLLAGGPSSGAPPPS

SEQ ID NO: 64 - protein, 39 aa, synthetic construct
  SITE 2: note = X is Aib
  MOD_RES 39: note = The C-terminal Ser is amidated
  SITE 16: note = X is a Lys, Orn, Dap, Dab, or Cys residue with the side chain linked to a substituent
HXHGTFTSDYSILLEXKAAQEFVEWLLAGGPSSGAPPPS

SEQ ID NO: 65 - protein, 39 aa, synthetic construct; identical to SEQ ID NO: 64
  SITE 2: note = X is Aib
  MOD_RES 39: note = The C-terminal Ser is amidated
  SITE 13: note = L is alpha-methyl-Leu
  SITE 16: note = X is a Lys, Orn, Dap, Dab, or Cys residue with the side chain linked to a substituent

SEQ ID NO: 66 - protein, 39 aa, synthetic construct
  SITE 2: note = X is Aib
  MOD_RES 39: note = The C-terminal Ser is amidated
  SITE 12: note = K is alpha-methyl-Lys
  SITE 20: note = S is alpha-methyl-Ser
  SITE 16: note = X is a Lys, Orn, Dap, Dab, or Cys residue with the side chain linked to a substituent
HXHGTFTSDYSKLLEXKAASEFVEWLIEGGPSSGAPPPS

SEQ ID NO: 67 - protein, 39 aa, synthetic construct
  SITE 2: note = X is Aib
  MOD_RES 39: note = The C-terminal Ser is amidated
  SITE 12: note = K is alpha-methyl-Lys
  SITE 20: note = X is isovaline
  SITE 16: note = X is a Lys, Orn, Dap, Dab, or Cys residue with the side chain linked to a substituent
YXQGTFTSDYSKLLEXKAAXEFVEWLLAGGPSSGAPPPS

SEQ ID NO: 68 - protein, 39 aa, synthetic construct
  SITE 2: note = X is Aib
  MOD_RES 39: note = The C-terminal Ser is amidated
  SITE 12: note = K is alpha-methyl-Lys
  SITE 20: note = X is isovaline
  SITE 16: note = X is a Lys, Orn, Dap, Dab, or Cys residue with the side chain linked to a substituent
HXHGTFTSDYSKLLEXQAAXEFVEWLLAGGPSSGAPPPS

SEQ ID NO: 69 - protein, 39 aa, synthetic construct
  SITE 2: note = X is Aib
  MOD_RES 39: note = The C-terminal Ser is amidated
  SITE 12: note = K is alpha-methyl-Lys
  SITE 20: note = X is isovaline
  SITE 16: note = X is a Lys, Orn, Dap, Dab, or Cys residue with the side chain linked to a substituent
YXQGTFTSDYSKILEXKAAXEFVEWLLAGGPSSGAPPPS

SEQ ID NO: 70 - protein, 39 aa, synthetic construct
  SITE 2: note = X is Aib
  MOD_RES 39: note = The C-terminal Ser is amidated
  SITE 12: note = K is alpha-methyl-Lys
  SITE 20: note = X is isovaline
  SITE 16: note = X is a Lys, Orn, Dap, Dab, or Cys residue with the side chain linked to a substituent
HXHGTFTSDYSKILEXQAAXEFVEWLLAGGPSSGAPPPS

SEQ ID NO: 71 - protein, 39 aa, synthetic construct
  SITE 2: note = X is Aib
  MOD_RES 39: note = The C-terminal Ser is amidated
  SITE 12: note = K is alpha-methyl-Lys
  SITE 20: note = X is isovaline
  SITE 16: note = X is a Lys, Orn, Dap, Dab, or Cys residue with the side chain linked to a substituent
HXHGTFTSDYSKLLEXKAAXEFVEWLIEGGPSSGAPPPS

SEQ ID NO: 72 - protein, 39 aa, synthetic construct
  SITE 2: note = X is Aib
  MOD_RES 39: note = The C-terminal Ser is amidated
  SITE 12: note = K is alpha-methyl-Lys
  SITE 20: note = X is isovaline
  SITE 16: note = X is a Lys, Orn, Dap, Dab, or Cys residue with the side chain linked to a substituent
HXHGTFTSDYSKILEXKAAXEFVEWLIEGGPSSGAPPPS

SEQ ID NO: 73 - protein, 39 aa, synthetic construct
  SITE 2: note = X is Aib
  MOD_RES 39: note = The C-terminal Ser is amidated
  SITE 12: note = K is alpha-methyl-Lys
  SITE 20: note = X is isovaline
  SITE 16: note = X is a Lys, Orn, Dap, Dab, or Cys residue with the side chain linked to a substituent
HXHGTFTSDLSKLLEXKAAXEFVEWLIEGGPSSGAPPPS

SEQ ID NO: 74 - protein, 39 aa, synthetic construct
  SITE 2: note = X is Aib
  MOD_RES 39: note = The C-terminal Ser is amidated
  SITE 12: note = K is alpha-methyl-Lys
  SITE 20: note = X is isovaline
  SITE 16: note = X is a Lys, Orn, Dap, Dab, or Cys residue with the side chain linked to a substituent
HXHGTFTSDLSKILEXKAAXEFVEWLIEGGPSSGAPPPS

SEQ ID NO: 75 - protein, 39 aa, synthetic construct
  SITE 2: note = X is Aib
  MOD_RES 39: note = The C-terminal Ser is amidated
  SITE 20: note = X is isovaline
  SITE 16: note = X is a Lys, Orn, Dap, Dab, or Cys residue with the side chain linked to a substituent
HXHGTFTSDYSILLEXKAAXEFVEWLLAGGPSSGAPPPS

SEQ ID NO: 76 - protein, 39 aa, synthetic construct
  SITE 2: note = X is Aib
  MOD_RES 39: note = The C-terminal Ser is amidated
  SITE 20: note = X is isovaline
  SITE 16: note = X is a Lys, Orn, Dap, Dab, or Cys residue with the side chain linked to a substituent
HXHGTFTSDLSILLEXKAAXEFVEWLLAGGPSSGAPPPS

SEQ ID NO: 77 - protein, 39 aa, synthetic construct; identical to SEQ ID NO: 75
  SITE 2: note = X is Aib
  MOD_RES 39: note = The C-terminal Ser is amidated
  SITE 13: note = L is alpha-methyl-Leu
  SITE 20: note = X is isovaline
  SITE 16: note = X is a Lys, Orn, Dap, Dab, or Cys residue with the side chain linked to a substituent

SEQ ID NO: 78 - protein, 39 aa, synthetic construct; identical to SEQ ID NO: 76
  SITE 2: note = X is Aib
  MOD_RES 39: note = The C-terminal Ser is amidated
  SITE 13: note = L is alpha-methyl-Leu
  SITE 20: note = X is isovaline
  SITE 16: note = X is a Lys, Orn, Dap, Dab, or Cys residue with the side chain linked to a substituent

SEQ ID NO: 79 - protein, 39 aa, synthetic construct
  SITE 2: note = X is Aib
  MOD_RES 39: note = The C-terminal Ser is amidated
  SITE 13: note = L is alpha-methyl-Leu
  SITE 29: note = E is D-Glu
  SITE 16: note = X is a Lys, Orn, Dap, Dab, or Cys residue with the side chain linked to a substituent
HXHGTFTSDYSILLEXKAAQEFVEWLLAEGPSSGAPPPS

SEQ ID NO: 80 - protein, 39 aa, synthetic construct; identical to SEQ ID NO: 76
  SITE 2: note = X is Aib
  MOD_RES 39: note = The C-terminal Ser is amidated
  SITE 13: note = L is alpha-methyl-Leu
  SITE 20: note = X is 1-aminocyclobutane-1-carboxylic acid
  SITE 16: note = X is a Lys, Orn, Dap, Dab, or Cys residue with the side chain linked to a substituent

SEQ ID NO: 81 - protein, 39 aa, synthetic construct
  SITE 2: note = X is Aib
  MOD_RES 39: note = The C-terminal Ser is amidated
  SITE 13: note = L is alpha-methyl-Leu
  SITE 29: note = E is D-Glu
  SITE 16: note = X is a Lys, Orn, Dap, Dab, or Cys residue with the side chain linked to a substituent
HXHGTFTSDLSILLEXKAAQEFVEWLLAEGPSSGAPPPS

SEQ ID NO: 82 - protein, 39 aa, synthetic construct
  SITE 2: note = X is Aib
  MOD_RES 39: note = The C-terminal Ser is amidated
  SITE 13: note = L is alpha-methyl-Leu
  SITE 16: note = X is a Lys, Orn, Dap, Dab, or Cys residue with the side chain linked to a substituent
HXHGTFTSDLSILLEXKAAQEFVEWLLAGGPSSGAPPPS

SEQ ID NO: 83 - protein, 39 aa, synthetic construct; identical to SEQ ID NO: 81
  SITE 2: note = X is Aib
  MOD_RES 39: note = The C-terminal Ser is amidated
  SITE 29: note = E is D-Glu
  SITE 16: note = X is a Lys, Orn, Dap, Dab, or Cys residue with the side chain linked to a substituent

SEQ ID NO: 84 - protein, 39 aa, synthetic construct
  SITE 2: note = X is Aib
  MOD_RES 39: note = The C-terminal Ser is amidated
  SITE 20: note = X is 1-aminocyclobutane-1-carboxylic acid
  SITE 29: note = E is D-Glu
  SITE 16: note = X is a Lys, Orn, Dap, Dab, or Cys residue with the side chain linked to a substituent
HXHGTFTSDLSILLEXQAAXEFVEWLLAEGPSSGAPPPS

SEQ ID NO: 85 - protein, 39 aa, synthetic construct
  SITE 2: note = X is Aib
  MOD_RES 39: note = The C-terminal Ser is amidated
  SITE 20: note = X is 1-aminocyclopropane-1-carboxylic acid
  SITE 29: note = E is D-Glu
  SITE 16: note = X is a Lys, Orn, Dap, Dab, or Cys residue with the side chain linked to a substituent
HXHGTFTSDLSILLEXKAAXEFVEWLLAEGPSSGAPPPS

SEQ ID NO: 86 - protein, 39 aa, synthetic construct; identical to SEQ ID NO: 85
  SITE 2: note = X is Aib
  MOD_RES 39: note = The C-terminal Ser is amidated
  SITE 20: note = X is 1-aminocyclobutane-1-carboxylic acid
  SITE 29: note = E is D-Glu
  SITE 16: note = X is a Lys, Orn, Dap, Dab, or Cys residue with the side chain linked to a substituent

SEQ ID NO: 87 - protein, 39 aa, synthetic construct; identical to SEQ ID NO: 84
  SITE 2: note = X is Aib
  MOD_RES 39: note = The C-terminal Ser is amidated
  SITE 20: note = X is 1-aminocyclopropane-1-carboxylic acid
  SITE 29: note = E is D-Glu
  SITE 16: note = X is a Lys, Orn, Dap, Dab, or Cys residue with the side chain linked to a substituent

SEQ ID NO: 88 - protein, 39 aa, synthetic construct
  SITE 2: note = X is Aib
  MOD_RES 39: note = The C-terminal Ser is amidated
  SITE 20: note = X is 1-aminocyclopropane-1-carboxylic acid
  SITE 29: note = E is D-Glu
  SITE 16: note = X is a Lys, Orn, Dap, Dab, or Cys residue with the side chain linked to a substituent
HXHGTFTSDYSILLEXQAAXEFVEWLLAEGPSSGAPPPS

SEQ ID NO: 89 - protein, 39 aa, synthetic construct; identical to SEQ ID NO: 88
  SITE 2: note = X is Aib
  MOD_RES 39: note = The C-terminal Ser is amidated
  SITE 20: note = X is 1-aminocyclobutane-1-carboxylic acid
  SITE 29: note = E is D-Glu
  SITE 16: note = X is a Lys, Orn, Dap, Dab, or Cys residue with the side chain linked to a substituent

SEQ ID NO: 90 - protein, 39 aa, synthetic construct; identical to SEQ ID NO: 79
  SITE 2: note = X is Aib
  MOD_RES 39: note = The C-terminal Ser is amidated
  SITE 29: note = E is D-Glu
  SITE 16: note = X is a Lys, Orn, Dap, Dab, or Cys residue with the side chain linked to a substituent

SEQ ID NO: 91 - protein, 39 aa, synthetic construct
  SITE 2: note = X is Aib
  MOD_RES 39: note = The C-terminal Ser is amidated
  SITE 16: note = X is a Lys, Orn, Dap, Dab, or Cys residue with the side chain linked to a substituent
HXHGTFTSDYSILLEXQAAQEFVEWLLAGGPSSGAPPPS

SEQ ID NO: 92 - protein, 39 aa, synthetic construct
  SITE 2: note = X is Aib
  MOD_RES 39: note = The C-terminal Ser is amidated
  SITE 29: note = E is D-Glu
  SITE 16: note = X is a Lys, Orn, Dap, Dab, or Cys residue with the side chain linked to a substituent
HXHGTFTSDYSILLEXQAAQEFVEWLLAEGPSSGAPPPS

SEQ ID NO: 93 - protein, 39 aa, synthetic construct
  SITE 2: note = X is Aib
  MOD_RES 39: note = The C-terminal Ser is amidated
  SITE 16: note = X is a Lys, Orn, Dap, Dab, or Cys residue with the side chain linked to a substituent
HXQGTFTSDYSILLEXKAAQEFVEWLLAGGPSSGAPPPS

SEQ ID NO: 94 - protein, 39 aa, synthetic construct; identical to SEQ ID NO: 93
  SITE 2: note = X is Aib
  MOD_RES 39: note = The C-terminal Ser is amidated
  SITE 13: note = L is alpha-methyl-Leu
  SITE 16: note = X is a Lys, Orn, Dap, Dab, or Cys residue with the side chain linked to a substituent

SEQ ID NO: 95 - protein, 39 aa, synthetic construct
  SITE 2: note = X is Aib
  MOD_RES 39: note = The C-terminal Ser is amidated
  SITE 20: note = X is Aib
  SITE 16: note = X is a Lys, Orn, Dap, Dab, or Cys residue with the side chain linked to a substituent
HXQGTFTSDYSILLEXKAAXEFVEWLLAGGPSSGAPPPS

SEQ ID NO: 96 - protein, 39 aa, synthetic construct; identical to SEQ ID NO: 95
  SITE 2: note = X is Aib
  MOD_RES 39: note = The C-terminal Ser is amidated
  SITE 13: note = L is alpha-methyl-Leu
  SITE 20: note = X is Aib
  SITE 16: note = X is a Lys, Orn, Dap, Dab, or Cys residue with the side chain linked to a substituent

SEQ ID NO: 97 - protein, 39 aa, synthetic construct; identical to SEQ ID NO: 1
  SITE 2: note = X is Aib
  SITE 12: note = K is alpha-methyl-Lys
  MOD_RES 39: note = The C-terminal Ser is amidated
  MOD_RES 17: note = The epsilon-amino group of the Lys residue is covalently linked to OEG-OEG-gammaGlu-C(O)-(CH2)18-COOH via an amide bond

SEQ ID NO: 98 - protein, 39 aa, synthetic construct; identical to SEQ ID NO: 2
  SITE 2: note = X is Aib
  SITE 12: note = K is alpha-methyl-Lys
  MOD_RES 39: note = The C-terminal Ser is amidated
  MOD_RES 16: note = The epsilon-amino group of the Lys residue is covalently linked to OEG-OEG-gammaGlu-C(O)-(CH2)18-COOH via an amide bond

SEQ ID NO: 99 - protein, 39 aa, synthetic construct; identical to SEQ ID NO: 2
  SITE 2: note = X is Aib
  SITE 13: note = Y is alpha-methyl-Tyr
  MOD_RES 39: note = The C-terminal Ser is amidated
  MOD_RES 16: note = The epsilon-amino group of the Lys residue is covalently linked to OEG-OEG-gammaGlu-C(O)-(CH2)18-COOH via an amide bond

SEQ ID NO: 100 - protein, 39 aa, synthetic construct; identical to SEQ ID NO: 4
  SITE 2: note = X is Aib
  SITE 13: note = X is Aib
  MOD_RES 39: note = The C-terminal Ser is amidated
  MOD_RES 16: note = The epsilon-amino group of the Lys residue is covalently linked to OEG-OEG-gammaGlu-C(O)-(CH2)18-COOH via an amide bond

SEQ ID NO: 101 - protein, 39 aa, synthetic construct; identical to SEQ ID NO: 2
  SITE 2: note = X is Aib
  SITE 14: note = L is alpha-methyl-Leu
  MOD_RES 39: note = The C-terminal Ser is amidated
  MOD_RES 16: note = The epsilon-amino group of the Lys residue is covalently linked to OEG-OEG-gammaGlu-C(O)-(CH2)18-COOH via an amide bond

SEQ ID NO: 102 - protein, 39 aa, synthetic construct; identical to SEQ ID NO: 2
  SITE 2: note = X is Aib
  SITE 17: note = K is alpha-methyl-Lys
  MOD_RES 39: note = The C-terminal Ser is amidated
  MOD_RES 16: note = The epsilon-amino group of the Lys residue is covalently linked to OEG-OEG-gammaGlu-C(O)-(CH2)18-COOH via an amide bond

SEQ ID NO: 103 - protein, 39 aa, synthetic construct; identical to SEQ ID NO: 7
  SITE 2: note = X is Aib
  SITE 18: note = X is Aib
  MOD_RES 39: note = The C-terminal Ser is amidated
  MOD_RES 16: note = The epsilon-amino group of the Lys residue is covalently linked to OEG-OEG-gammaGlu-C(O)-(CH2)18-COOH via an amide bond

SEQ ID NO: 104 - protein, 39 aa, synthetic construct; identical to SEQ ID NO: 8
  SITE 2: note = X is Aib
  MOD_RES 39: note = The C-terminal Ser is amidated
  SITE 12: note = K is alpha-methyl-Lys
  MOD_RES 16: note = The epsilon-amino group of the Lys residue is covalently linked to OEG-OEG-gammaGlu-C(O)-(CH2)18-COOH via an amide bond

SEQ ID NO: 105 - protein, 39 aa, synthetic construct; identical to SEQ ID NO: 9
  SITE 2: note = X is Aib
  MOD_RES 39: note = The C-terminal Ser is amidated
  SITE 12: note = K is alpha-methyl-Lys
  MOD_RES 16: note = The epsilon-amino group of the Lys residue is covalently linked to OEG-OEG-gammaGlu-C(O)-(CH2)18-COOH via an amide bond

SEQ ID NO: 106 - protein, 39 aa, synthetic construct; identical to SEQ ID NO: 10
  SITE 2: note = X is Aib
  MOD_RES 39: note = The C-terminal Ser is amidated
  SITE 12: note = K is alpha-methyl-Lys
  MOD_RES 16: note = The epsilon-amino group of the Lys residue is covalently linked to OEG-OEG-gammaGlu-C(O)-(CH2)18-COOH via an amide bond

SEQ ID NO: 107 - protein, 39 aa, synthetic construct; identical to SEQ ID NO: 11
  SITE 2: note = X is Aib
  MOD_RES 39: note = The C-terminal Ser is amidated
  SITE 12: note = K is alpha-methyl-Lys
  MOD_RES 16: note = The epsilon-amino group of the Lys residue is covalently linked to OEG-OEG-gammaGlu-C(O)-(CH2)18-COOH via an amide bond

SEQ ID NO: 108 - protein, 39 aa, synthetic construct; identical to SEQ ID NO: 12
  SITE 2: note = X is Aib
  MOD_RES 39: note = The C-terminal Ser is amidated
  SITE 12: note = K is alpha-methyl-Lys
  MOD_RES 16: note = The epsilon-amino group of the Lys residue is covalently linked to OEG-OEG-gammaGlu-C(O)-(CH2)18-COOH via an amide bond

SEQ ID NO: 109 - protein, 39 aa, synthetic construct; identical to SEQ ID NO: 13
  SITE 2: note = X is Aib
  MOD_RES 39: note = The C-terminal Ser is amidated
  SITE 12: note = K is alpha-methyl-Lys
  MOD_RES 16: note = The epsilon-amino group of the Lys residue is covalently linked to OEG-OEG-gammaGlu-C(O)-(CH2)18-COOH via an amide bond

SEQ ID NO: 110 - protein, 39 aa, synthetic construct; identical to SEQ ID NO: 14
  SITE 2: note = X is Aib
  MOD_RES 39: note = The C-terminal Ser is amidated
  SITE 12: note = K is alpha-methyl-Lys
  MOD_RES 16: note = The epsilon-amino group of the Lys residue is covalently linked to OEG-OEG-gammaGlu-C(O)-(CH2)18-COOH via an amide bond

SEQ ID NO: 111 - protein, 39 aa, synthetic construct; identical to SEQ ID NO: 15
  SITE 2: note = X is Aib
  MOD_RES 39: note = The C-terminal Ser is amidated
  SITE 12: note = K is alpha-methyl-Lys
  MOD_RES 16: note = The epsilon-amino group of the Lys residue is covalently linked to OEG-OEG-gammaGlu-C(O)-(CH2)18-COOH via an amide bond

SEQ ID NO: 112 - protein, 39 aa, synthetic construct; identical to SEQ ID NO: 16
  SITE 2: note = X is Aib
  MOD_RES 39: note = The C-terminal Ser is amidated
  MOD_RES 16: note = The epsilon-amino group of the Lys residue is covalently linked to OEG-OEG-gammaGlu-C(O)-(CH2)18-COOH via an amide bond

SEQ ID NO: 113 - protein, 39 aa, synthetic construct; identical to SEQ ID NO: 16
  SITE 2: note = X is Aib
  MOD_RES 39: note = The C-terminal Ser is amidated
  SITE 13: note = L is alpha-methyl-Leu
  MOD_RES 16: note = The epsilon-amino group of the Lys residue is covalently linked to OEG-OEG-gammaGlu-C(O)-(CH2)18-COOH via an amide bond

SEQ ID NO: 114 - protein, 39 aa, synthetic construct; identical to SEQ ID NO: 18
  SITE 2: note = X is Aib
  MOD_RES 39: note = The C-terminal Ser is amidated
  SITE 12: note = K is alpha-methyl-Lys
  SITE 20: note = S is alpha-methyl-Ser
  MOD_RES 16: note = The epsilon-amino group of the Lys residue is covalently linked to OEG-OEG-gammaGlu-C(O)-(CH2)18-COOH via an amide bond

SEQ ID NO: 115 - protein, 39 aa, synthetic construct; identical to SEQ ID NO: 19
  SITE 2: note = X is Aib
  MOD_RES 39: note = The C-terminal Ser is amidated
  SITE 12: note = K is alpha-methyl-Lys
  SITE 20: note = X is isovaline
  MOD_RES 16: note = The epsilon-amino group of the Lys residue is covalently linked to OEG-OEG-gammaGlu-C(O)-(CH2)18-COOH via an amide bond

SEQ ID NO: 116 - protein, 39 aa, synthetic construct; identical to SEQ ID NO: 20
  SITE 2: note = X is Aib
  MOD_RES 39: note = The C-terminal Ser is amidated
  SITE 12: note = K is alpha-methyl-Lys
  SITE 20: note = X is isovaline
  MOD_RES 16: note = The epsilon-amino group of the Lys residue is covalently linked to OEG-OEG-gammaGlu-C(O)-(CH2)18-COOH via an amide bond

SEQ ID NO: 117 - protein, 39 aa, synthetic construct; identical to SEQ ID NO: 21
  SITE 2: note = X is Aib
  MOD_RES 39: note = The C-terminal Ser is amidated
  SITE 12: note = K is alpha-methyl-Lys
  SITE 20: note = X is isovaline
  MOD_RES 16: note = The epsilon-amino group of the Lys residue is covalently linked to OEG-OEG-gammaGlu-C(O)-(CH2)18-COOH via an amide bond

SEQ ID NO: 118 - protein, 39 aa, synthetic construct; identical to SEQ ID NO: 22
  SITE 2: note = X is Aib
  MOD_RES 39: note = The C-terminal Ser is amidated
  SITE 12: note = K is alpha-methyl-Lys
  SITE 20: note = X is isovaline
  MOD_RES 16: note = The epsilon-amino group of the Lys residue is covalently linked to OEG-OEG-gammaGlu-C(O)-(CH2)18-COOH via an amide bond

SEQ ID NO: 119 - protein, 39 aa, synthetic construct; identical to SEQ ID NO: 23
  SITE 2: note = X is Aib
  MOD_RES 39: note = The C-terminal Ser is amidated
  SITE 12: note = K is alpha-methyl-Lys
  SITE 20: note = X is isovaline
  MOD_RES 16: note = The epsilon-amino group of the Lys residue is covalently linked to OEG-OEG-gammaGlu-C(O)-(CH2)18-COOH via an amide bond

SEQ ID NO: 120 - protein, 39 aa, synthetic construct; identical to SEQ ID NO: 24
  SITE 2: note = X is Aib
  MOD_RES 39: note = The C-terminal Ser is amidated
  SITE 12: note = K is alpha-methyl-Lys
  SITE 20: note = X is isovaline
  MOD_RES 16: note = The epsilon-amino group of the Lys residue is covalently linked to OEG-OEG-gammaGlu-C(O)-(CH2)18-COOH via an amide bond

SEQ ID NO: 121 - protein, 39 aa, synthetic construct; identical to SEQ ID NO: 25
  SITE 2: note = X is Aib
  MOD_RES 39: note = The C-terminal Ser is amidated
  SITE 12: note = K is alpha-methyl-Lys
  SITE 20: note = X is isovaline
  MOD_RES 16: note = The epsilon-amino group of the Lys residue is covalently linked to OEG-OEG-gammaGlu-C(O)-(CH2)18-COOH via an amide bond

SEQ ID NO: 122 - protein, 39 aa, synthetic construct; identical to SEQ ID NO: 26
  SITE 2: note = X is Aib
  MOD_RES 39: note = The C-terminal Ser is amidated
  SITE 12: note = K is alpha-methyl-Lys
  SITE 20: note = X is isovaline
  MOD_RES 16: note = The epsilon-amino group of the Lys residue is covalently linked to OEG-OEG-gammaGlu-C(O)-(CH2)18-COOH via an amide bond

SEQ ID NO: 123 - protein, 39 aa, synthetic construct; identical to SEQ ID NO: 27
  SITE 2: note = X is Aib
  MOD_RES 39: note = The C-terminal Ser is amidated
  SITE 20: note = X is isovaline
  MOD_RES 16: note = The epsilon-amino group of the Lys residue is covalently linked to OEG-OEG-gammaGlu-C(O)-(CH2)18-COOH via an amide bond

SEQ ID NO: 124 - protein, 39 aa, synthetic construct; identical to SEQ ID NO: 28
  SITE 2: note = X is Aib
  MOD_RES 39: note = The C-terminal Ser is amidated
  SITE 20: note = X is isovaline
  MOD_RES 16: note = The epsilon-amino group of the Lys residue is covalently linked to OEG-OEG-gammaGlu-C(O)-(CH2)18-COOH via an amide bond

SEQ ID NO: 125 - protein, 39 aa, synthetic construct; identical to SEQ ID NO: 27
  SITE 2: note = X is Aib
  MOD_RES 39: note = The C-terminal Ser is amidated
  SITE 13: note = L is alpha-methyl-Leu
  SITE 20: note = X is isovaline
  MOD_RES 16: note = The epsilon-amino group of the Lys residue is covalently linked to OEG-OEG-gammaGlu-C(O)-(CH2)18-COOH via an amide bond

SEQ ID NO: 126 - protein, 39 aa, synthetic construct; identical to SEQ ID NO: 28
  SITE 2: note = X is Aib
  MOD_RES 39: note = The C-terminal Ser is amidated
  SITE 13: note = L is alpha-methyl-Leu
  SITE 20: note = X is isovaline
  MOD_RES 16: note = The epsilon-amino group of the Lys residue is covalently linked to OEG-OEG-gammaGlu-C(O)-(CH2)18-COOH via an amide bond

SEQ ID NO: 127 - protein, 39 aa, synthetic construct; identical to SEQ ID NO: 31
  SITE 2: note = X is Aib
  MOD_RES 39: note = The C-terminal Ser is amidated
  SITE 13: note = L is alpha-methyl-Leu
  SITE 29: note = E is D-Glu
  MOD_RES 16: note = The epsilon-amino group of the Lys residue is covalently linked to OEG-OEG-gammaGlu-C(O)-(CH2)18-COOH via an amide bond

SEQ ID NO: 128 - protein, 39 aa, synthetic construct; identical to SEQ ID NO: 28
  SITE 2: note = X is Aib
  MOD_RES 39: note = The C-terminal Ser is amidated
  SITE 13: note = L is alpha-methyl-Leu
  SITE 20: note = X is 1-aminocyclobutane-1-carboxylic acid
  MOD_RES 16: note = The epsilon-amino group of the Lys residue is covalently linked to OEG-OEG-gammaGlu-C(O)-(CH2)18-COOH via an amide bond

SEQ ID NO: 129 - protein, 39 aa, synthetic construct; identical to SEQ ID NO: 33
  SITE 2: note = X is Aib
  MOD_RES 39: note = The C-terminal Ser is amidated
  SITE 13: note = L is alpha-methyl-Leu
  SITE 29: note = E is D-Glu
  MOD_RES 16: note = The epsilon-amino group of the Lys residue is covalently linked to OEG-OEG-gammaGlu-C(O)-(CH2)18-COOH via an amide bond

SEQ ID NO: 130 - protein, 39 aa, synthetic construct; identical to SEQ ID NO: 34
  SITE 2: note = X is Aib
  MOD_RES 39: note = The C-terminal Ser is amidated
  SITE 13: note = L is alpha-methyl-Leu
  MOD_RES 16: note = The epsilon-amino group of the Lys residue is covalently linked to OEG-OEG-gammaGlu-C(O)-(CH2)18-COOH via an amide bond

SEQ ID NO: 131 - protein, 39 aa, synthetic construct; identical to SEQ ID NO: 33
  SITE 2: note = X is Aib
  MOD_RES 39: note = The C-terminal Ser is amidated
  SITE 29: note = E is D-Glu
  MOD_RES 16: note = The epsilon-amino group of the Lys residue is covalently linked to OEG-OEG-gammaGlu-C(O)-(CH2)18-COOH via an amide bond

SEQ ID NO: 132 - protein, 39 aa, synthetic construct; identical to SEQ ID NO: 36
  SITE 2: note = X is Aib
  MOD_RES 39: note = The C-terminal Ser is amidated
  SITE 20: note = X is 1-aminocyclobutane-1-carboxylic acid
  SITE 29: note = E is D-Glu
  MOD_RES 16: note = The epsilon-amino group of the Lys residue is covalently linked to OEG-OEG-gammaGlu-C(O)-(CH2)18-COOH via an amide bond

SEQ ID NO: 133 - protein, 39 aa, synthetic construct; identical to SEQ ID NO: 37
  SITE 2: note = X is Aib
  MOD_RES 39: note = The C-terminal Ser is amidated
  SITE 20: note = X is 1-aminocyclopropane-1-carboxylic acid
  SITE 29: note = E is D-Glu
  MOD_RES 16: note = The epsilon-amino group of the Lys residue is covalently linked to OEG-OEG-gammaGlu-C(O)-(CH2)18-COOH via an amide bond

SEQ ID NO: 134 - protein, 39 aa, synthetic construct; identical to SEQ ID NO: 37
  SITE 2: note = X is Aib
  MOD_RES 39: note = The C-terminal Ser is amidated
  SITE 20: note = X is 1-aminocyclobutane-1-carboxylic acid
  SITE 29: note = E is D-Glu
  MOD_RES 16: note = The epsilon-amino group of the Lys residue is covalently linked to OEG-OEG-gammaGlu-C(O)-(CH2)18-COOH via an amide bond

SEQ ID NO: 135 - protein, 39 aa, synthetic construct; identical to SEQ ID NO: 36
  SITE 2: note = X is Aib
  MOD_RES 39: note = The C-terminal Ser is amidated
  SITE 20: note = X is 1-aminocyclopropane-1-carboxylic acid
  SITE 29: note = E is D-Glu
  MOD_RES 16: note = The epsilon-amino group of the Lys residue is covalently linked to OEG-OEG-gammaGlu-C(O)-(CH2)18-COOH via an amide bond

SEQ ID NO: 136 - protein, 39 aa, synthetic construct; identical to SEQ ID NO: 40
  SITE 2: note = X is Aib
  MOD_RES 39: note = The C-terminal Ser is amidated
  SITE 20: note = X is 1-aminocyclopropane-1-carboxylic acid
  SITE 29: note = E is D-Glu
  MOD_RES 16: note = The epsilon-amino group of the Lys residue is covalently linked to OEG-OEG-gammaGlu-C(O)-(CH2)18-COOH via an amide bond

SEQ ID NO: 137 - protein, 39 aa, synthetic construct; identical to SEQ ID NO: 40
  SITE 2: note = X is Aib
  MOD_RES 39: note = The C-terminal Ser is amidated
  SITE 20: note = X is 1-aminocyclobutane-1-carboxylic acid
  SITE 29: note = E is D-Glu
  MOD_RES 16: note = The epsilon-amino group of the Lys residue is covalently linked to OEG-OEG-gammaGlu-C(O)-(CH2)18-COOH via an amide bond

SEQ ID NO: 138 - protein, 39 aa, synthetic construct; identical to SEQ ID NO: 31
  SITE 2: note = X is Aib
  MOD_RES 39: note = The C-terminal Ser is amidated
  SITE 29: note = E is D-Glu
  MOD_RES 16: note = The epsilon-amino group of the Lys residue is covalently linked to OEG-OEG-gammaGlu-C(O)-(CH2)18-COOH via an amide bond

SEQ ID NO: 139 - protein, 39 aa, synthetic construct; identical to SEQ ID NO: 43
  SITE 2: note = X is Aib
  MOD_RES 39: note = The C-terminal Ser is amidated
  MOD_RES 16: note = The epsilon-amino group of the Lys residue is covalently linked to OEG-OEG-gammaGlu-C(O)-(CH2)18-COOH via an amide bond

SEQ ID NO: 140 - protein, 39 aa, synthetic construct; identical to SEQ ID NO: 44
  SITE 2: note = X is Aib
  MOD_RES 39: note = The C-terminal Ser is amidated
  SITE 29: note = E is D-Glu
  MOD_RES 16: note = The epsilon-amino group of the Lys residue is covalently linked to OEG-OEG-gammaGlu-C(O)-(CH2)18-COOH via an amide bond

SEQ ID NO: 141 - protein, 39 aa, synthetic construct; identical to SEQ ID NO: 45
  SITE 2: note = X is Aib
  MOD_RES 39: note = The C-terminal Ser is amidated
  MOD_RES 16: note = The epsilon-amino group of the Lys residue is covalently linked to OEG-OEG-gammaGlu-C(O)-(CH2)18-COOH via an amide bond

SEQ ID NO: 142 - protein, 39 aa, synthetic construct; identical to SEQ ID NO: 45
  SITE 2: note = X is Aib
  MOD_RES 39: note = The C-terminal Ser is amidated
  SITE 13: note = L is alpha-methyl-Leu
  MOD_RES 16: note = The epsilon-amino group of the Lys residue is covalently linked to OEG-OEG-gammaGlu-C(O)-(CH2)18-COOH via an amide bond

SEQ ID NO: 143 - protein, 39 aa, synthetic construct; identical to SEQ ID NO: 47
  SITE 2: note = X is Aib
  MOD_RES 39: note = The C-terminal Ser is amidated
  SITE 20: note = X is Aib
  MOD_RES 16: note = The epsilon-amino group of the Lys residue is covalently linked to OEG-OEG-gammaGlu-C(O)-(CH2)18-COOH via an amide bond

SEQ ID NO: 144 - protein, 39 aa, synthetic construct; identical to SEQ ID NO: 47
  SITE 2: note = X is Aib
  MOD_RES 39: note = The C-terminal Ser is amidated
  SITE 13: note = L is alpha-methyl-Leu
  SITE 20: note = X is Aib
  MOD_RES 16: note = The epsilon-amino group of the Lys residue is covalently linked to OEG-OEG-gammaGlu-C(O)-(CH2)18-COOH via an amide bond

SEQ ID NO: 145 - protein, 31 aa, synthetic construct
  SITE 1: note = X1 is selected from any natural amino acids, unnatural amino acids, or peptide segments composed of natural amino acids and/or unnatural amino acids
  SITE 2: note = X2 is selected from any natural amino acids, unnatural amino acids, or peptide segments composed of natural amino acids and/or unnatural amino acids
  SITE 3: note = X3 is selected from any natural amino acids, unnatural amino acids, or peptide segments composed of natural amino acids and/or unnatural amino acids
  SITE 10: note = X10 is selected from any natural amino acids, unnatural amino acids, or peptide segments composed of natural amino acids and/or unnatural amino acids
  SITE 12: note = X12 is selected from any natural amino acids, unnatural amino acids, or peptide segments composed of natural amino acids and/or unnatural amino acids
  SITE 13: note = X2 is selected from any natural amino acids, unnatural amino acids, or peptide segments composed of natural amino acids and/or unnatural amino acids
  SITE 14: note = X14 is selected from any natural amino acids, unnatural amino acids, or peptide segments composed of natural amino acids and/or unnatural amino acids
  SITE 16: note = X16 is selected from any natural amino acids, unnatural amino acids, or peptide segments composed of natural amino acids and/or unnatural amino acids
  SITE 17: note = X17 is selected from any natural amino acids, unnatural amino acids, or peptide segments composed of natural amino acids and/or unnatural amino acids
  SITE 18: note = X18 is selected from any natural amino acids, unnatural amino acids, or peptide segments composed of natural amino acids and/or unnatural amino acids
  SITE 19: note = X19 is selected from any natural amino acids, unnatural amino acids, or peptide segments composed of natural amino acids and/or unnatural amino acids
  SITE 20: note = X20 is selected from any natural amino acids, unnatural amino acids, or peptide segments composed of natural amino acids and/or unnatural amino acids
  SITE 21: note = X21 is selected from any natural amino acids, unnatural amino acids, or peptide segments composed of natural amino acids and/or unnatural amino acids
  SITE 27: note = X27 is selected from any natural amino acids, unnatural amino acids, or peptide segments composed of natural amino acids and/or unnatural amino acids
  SITE 28: note = X28 is selected from any natural amino acids, unnatural amino acids, or peptide segments composed of natural amino acids and/or unnatural amino acids
  SITE 29: note = X29 is selected from any natural amino acids, unnatural amino acids, or peptide segments composed of natural amino acids and/or unnatural amino acids
  SITE 30: note = Z is selected from any natural amino acids, unnatural amino acids, or peptide segments composed of natural amino acids and/or unnatural amino acids
  SITE 31: note = X40 is selected from any natural amino acids, unnatural amino acids, or peptide segments composed of natural amino acids and/or unnatural amino acids
XXXGTFTSDXSXXXEXXXXXXFVEWLXXXXX

SEQ ID NO: 146 - protein, 10 aa, synthetic construct
GPSSGAPPPS

SEQ ID NO: 147 - protein, 9 aa, synthetic construct
GPSSGAPPS

SEQ ID NO: 148 - protein, 9 aa, synthetic construct
PSSGAPPPS

SEQ ID NO: 149 - protein, 8 aa, synthetic construct
PSSGAPPS

SEQ ID NO: 150 - protein, 39 aa, synthetic construct
  SITE 1: note = X1 is selected from an amino acid residue of Tyr or His
  SITE 2: note = X2 is an amino acid residue of Aib
  SITE 3: note = X3 is selected from an amino acid residue of Gln or His
  SITE 10: note = X10 is selected from an amino acid residue of Leu or Tyr
  SITE 12: note = X12 is selected from an amino acid residue of Lys, alpha-methyl-Lys, or Ile
  SITE 13: note = X13 is selected from an amino acid residue of Aib, Ile, Leu, Tyr, alpha-methyl-Tyr or alpha-methyl-Leu
  SITE 14: note = X14 is selected from an amino acid residue of Leu or alpha-methyl-Leu
  SITE 17: note = X17 is selected from an amino acid residue of Ile, Lys, Gln, or alpha-methyl-Lys
  SITE 18: note = X18 is selected from an amino acid residue of Ala or Aib
  SITE 19: note = X19 is selected from an amino acid residue of Ala or Gln
  SITE 20: note = X20 is selected from an amino acid residue of Gln, Aib, isovaline, alpha-methyl-Ser, 1-aminocyclopropane-1-carboxylic acid or 1-aminocyclobutane-1-carboxylic acid
  SITE 27: note = X27 is selected from an amino acid residue of Ile or Leu
  SITE 28: note = X28 is selected from an amino acid residue of Ala or Glu
  SITE 29: note = X29 is selected from an amino acid residue of Gly or D-Glu
  SITE 16: note = Y1 is a Lys, Orn, Dap, Dab, or Cys residue with the side chain linked to a substituent
XXXGTFTSDXSXXXEXXXXXEFVEWLXXXGPSSGAPPPS

SEQ ID NO: 151 - protein, 33 aa, synthetic construct
  SITE 1: note = X1 is selected from an amino acid residue of Tyr or His
  SITE 2: note = X2 is an amino acid residue of Aib
  SITE 3: note = X3 is selected from an amino acid residue of Gln or His
  SITE 10: note = X10 is selected from an amino acid residue of Leu or Tyr
  SITE 12: note = X12 is selected from an amino acid residue of Lys, alpha-methyl-Lys, or Ile
  SITE 13: note = X13 is selected from an amino acid residue of Aib, Ile, Leu, Tyr, alpha-methyl-Tyr or alpha-methyl-Leu
  SITE 14: note = X14 is selected from an amino acid residue of Leu or alpha-methyl-Leu
  SITE 17: note = X17 is selected from an amino acid residue of Glu, Arg, homoArg, Ile, Lys, Gln, or alpha-methyl-Lys
  SITE 18: note = X18 is selected from an amino acid residue of Ala or Aib
  SITE 19: note = X19 is selected from an amino acid residue of Ala or Gln
  SITE 20: note = X20 is selected from an amino acid residue of Gln, Aib, isovaline, alpha-methyl-Ser, 1-aminocyclopropane-1-carboxylic acid or 1-aminocyclobutane-1-carboxylic acid
  SITE 27: note = X27 is selected from an amino acid residue of Ile or Leu
  SITE 28: note = X28 is selected from an amino acid residue of Ala or Glu
  SITE 29: note = X29 is selected from an amino acid residue of Gly or D-Glu
  SITE 31: note = X40 is selected from an amino acid residue of Lys, or is absent
  SITE 30: note = Z is selected from Gly-Pro-Ser-Ser-Gly-Ala-Pro-Pro-Pro-Ser, Gly-Pro-Ser-Ser-Gly-Ala-Pro-Pro-Ser, Pro-Ser-Ser-Gly-Ala-Pro-Pro-Pro-Ser, or Pro-Ser-Ser-Gly-Ala-Pro-Pro-Ser
  SITE 16: note = Y1 is a Lys, Orn, Dap, Dab, or Cys residue with the side chain linked to a substituent having the structure shown below: -Z1-Z2, wherein Z1 comprises 0-10 amino acid residues independently selected from Gly, Glu, gammaGlu, and OEG ([2-(2-amino-ethoxy)-ethoxy]-acetyl), and Z2 is selected from C12-32 fatty acids
XXXGTFTSDXSERXXXEXXXXXEFVEWLXXXXX